European Patent Application EP 4 317 430 A1, published February 7, 2024. Title: Method for Improving Efficiency of Genetic Transformation and Gene Editing in Plants. Applicant: Suzhou Qi Biodesign biotechnology Company Limited. The sequence listing filed with the application follows.

SEQUENCE LISTING (6 sequences)

SEQ ID NO: 1 - protein, 582 aa, Fragaria x ananassa
MSSFGFLSPPPISSSAPTRQLSAATTPAAAPIVAPDVAAERLEPRVEERQGYWVLKEKFRQGINVQEKVKIQREPMKLYMEGGIEELAKLPFEELDKAKDTKDDIDVRLKWLGLFHRRKHHYGRFMMRLKLPNGVTTSAQTRYLASVIRRYGKDGCADVTTRQNWQIRGIVLADVPDILKGLAGVGLTSLQSGMDNVRNPVGNPLAGIDPHEIVDTRPYTNLLSQYITGNSLGNPTITNLPRKWNVCVIGSHDLYEHPHINDLAYMPATKDGKFGFNLLVGGFFSPKRCAEAVPLDAWVSTEDMIPVCKAILEAYRDLGFRGNRQKTRMMWLIDELGIEGFRSEVVKRMPFKELERASTEDLVQKQWERRDYIGVHPQKQEGLSFVGLHIPVGRIQADDMDELARIADEYGTGELRLTVEQNIIIPNVENTKLQALLQEPLLKEKFSPEPSILMKGLVACTGNQFCGQAIIETKQRALKVTEEVERHVSVTRPVRMHWTGCPNTCGQVQVADIGFMGCMARDENGKPVEGVDVFLGGRIGSDSHLGDIYKKSVPCKDLVPLVIDILVNHFGAVPREREEGEE

SEQ ID NO: 2 - DNA, 1749 bp, Fragaria x ananassa
atgtcgtcatttgggttcctatctcctcctcctatatcctcctcggctcccacgaggcagctctccgcagccactactccggctgcggcaccgattgtcgctccggacgtggctgcggagaggctggagccgagggtggaggagagacaagggtattgggtgttgaaggagaagtttcgacaagggattaatgttcaggagaaggtcaagattcagagggagcctatgaagctatatatggaaggcgggattgaagagcttgctaagttgccttttgaggagcttgacaaagctaaggatactaaggatgatattgatgttaggctcaagtggcttggtctcttccacagaagaaagcatcactatggtagatttatgatgaggctgaagcttccgaatggggtcacaacaagtgcacagacaagatatctagcgagtgtgatacggagatatggcaaggatggttgtgcagatgtgacaaccaggcaaaattggcaaatccgcggaattgtgctggcagatgtgcctgatattctgaagggtcttgctggagtaggattgactagtctgcagagtgggatggacaatgtgagaaacccagttgggaatccacttgcaggcattgacccgcatgaaattgttgacacaagaccttacacgaacttgttgtcccaatacattactggcaattcactcggcaatccaactataacaaacttgccaaggaagtggaatgtgtgtgtgatagggtctcatgatctttatgagcatccccacatcaatgatcttgcgtacatgcctgcaacaaaggatgggaaatttggattcaatttactcgttggaggcttcttcagtcccaaaagatgtgcagaggcagttcctcttgatgcatgggtctcaactgaagatatgatcccagtttgcaaagctattctagaggcttatagagaccttggattcagaggcaaccgacaaaagacaagaatgatgtggttgatcgatgaactaggcatagaaggattcagatcagaggttgttaagagaatgccctttaaggaactggaaagagcatctactgaagacttggtacagaagcaatgggaaaggagagactatataggtgtccatccacagaaacaagaaggtctaagctttgtgggtcttcacattcccgtaggcaggatccaagcagatgacatggatgagctagctcgtatagctgacgagtatggcactggggaactccgtctcactgtggagcaaaacattattatccccaatgttgagaacacgaaactccaagcattgcttcaagaaccgcttctgaaagaaaaattttcacctgaaccttccattctcatgaaaggactagtagcttgcactggcaaccagttttgcggccaagccatcatcgagacaaagcaacgggccttgaaggtgactgaggaggtggaaaggcatgtgtcagtgactcggccagtgaggatgcattggacggggtgccccaatacctgcgggcaggtgcaagtggcagatataggtttcatggggtgtatggcaagggatgagaatggaaagcctgttgaaggggttgatgtcttcttgggaggaagaataggaagtgactctcatttgggagatatttataagaagagtgtcccttgtaaggacttggtgcccttagttattgacatcttggtaaatcactttggggctgtcccaagggagagggaagaaggggaagagtaa

SEQ ID NO: 3 - protein, 506 aa, Triticum aestivum
MALFTEGGIKELAKLPMEQIDADKLTKEDVDVRLKWLGLFHRRKQQYGRFMMRLKLPNGVTTSEQTRYLAGVIEKYGKEGCADVTTRQNWQIRGVTLPDVPEILEGLRSVGLTSLQSGMDNVRNPVGSPLAGIDPLEIVDTRPYTNLLSSYITNNSEGNLAITNLPRKWNVCVIGTHDLYEHPHINDLAYMPAEKDGKFGFNLLVGGFISPKRWGEALPLDAWVPGDDIIPVCKAVLEAFRDLGTRGNRQKTRMMWLIDELGMEAFRSEIEKRMPNGVLERAAAEDLIDKKWERRDYLGVHPQKQEGLSFVGLHVPVGRLQAADMFELARLADEYGSGELRLTVEQNIVLPNVKNEKVEALLAEPLLQKFSAHPSLLMKGLVACTGNQFCGQAIIETKARALQVTRDVEARVSVPRAVRMHWTGCPNSCAQVQVADIGFMGCLTKNSSGKIVEAADIFVGGRVGSDSHLTGVYKKAVPCEDLVPLVADLLVERFGAVPREREEDEE

SEQ ID NO: 4 - DNA, 1521 bp, Triticum aestivum
atggcgctcttcacggagggcggcatcaaggagctcgccaagctgcccatggagcagatcgacgccgacaagctcaccaaggaggacgtcgacgtgcggctcaagtggctcggcctcttccaccgccgcaagcagcagtatgggcggttcatgatgcggctgaagctgcccaacggcgtgacgacgagcgagcagacgcgctacctggccggcgtgatcgagaagtacggcaaggaggggtgcgccgacgtgacgacccggcagaactggcagatccgcggcgtgacgctgccggacgtgccggagatcctggaggggctccgctccgttggcctcaccagcctgcagagcggcatggacaacgtgcgcaaccccgtcggcagcccgctcgccggcatcgaccccctcgagatcgtcgacacgcgcccctacaccaacctcctctcctcctacatcaccaacaactccgagggcaacctcgccatcaccaaccttcctaggaagtggaacgtgtgcgtgatcggtacccatgacctgtacgagcacccgcacatcaacgacctggcgtacatgccggccgagaaggacggcaagttcgggttcaacctgctggtgggcgggttcatcagccccaagaggtggggcgaggccctgccgctcgacgcctgggtccccggcgacgacatcatcccggtctgcaaggccgtcctcgaggctttccgcgacctcggcaccaggggcaaccgccagaagacgcgcatgatgtggctcatcgacgagctcgggatggaggcgttccggtcggagatcgagaagaggatgccgaacggcgtgctggagcgcgcggcggccgaggacctgatcgacaagaagtgggagcggcgcgactacctcggcgtgcacccgcagaagcaggaggggctctccttcgtgggcctgcacgtgcccgtcggccggctgcaggccgccgacatgttcgagctggcccgcctcgccgacgagtacggctccggcgagctccgcctcaccgtggagcagaacatcgtcctccccaacgtcaagaacgagaaggtggaagctctgctcgccgagccgctgctgcagaagttctcggcgcacccgtcgctgctgatgaaggggctggtggcgtgcacgggcaaccagttctgcgggcaggccatcatcgagaccaaggcgcgggcgctgcaggtgacgcgcgacgtggaggcgcgcgtgtccgtgcccagggcggtgcgcatgcactggacggggtgccccaacagctgcgcgcaggtgcaggtggccgacatcggcttcatgggctgcctcaccaagaacagcagcggcaagatcgtcgaggcggcggacatcttcgtcggcggccgcgtcggcagcgactcgcacctcaccggggtgtacaagaaggcggtgccgtgcgaggacctggtgcccctcgtcgccgacctcctggtggagcggttcggggccgtgcccagggagagggaggaggacgaggagtag

SEQ ID NO: 5 - protein, 587 aa, Solanum lycopersicum
MASFSIKFLAPSLPNPTRFSKSSIVKLNATPPQTVAAAGPPEVAAERLEPRVEEKDGYWILKEQFRQGINPQEKVKIEKEPMKLFMENGIEELAKIPIEEIDQSKLTKDDIDVRLKWLGLFHRRKNQYGRFMMRLKLPNGVTTSAQTRYLASVIRKYGEEGCADITTRQNWQIRGVVLPDVPEILKGLEEVGLTSLQSGMDNVRNPVGNPLAGIDPEEIVDTRPYTNLLSQFITGNSRGNPAVSNLPRKWNPCVVGSHDLYEHPHINDLAYMPAIKDGRFGFNLLVGGFFSAKRCDEAIPLDAWVPADDVVPVCKAILEAFRDLGFRGNRQKCRMMWLIDELGVEGFRAEVVKRMPQQELERASPEDLVQKQWERRDYLGVHPQKQEGYSFIGLHIPVGRVQADDMDDLARLADEYGSGELRLTVEQNIIIPNIENSKIDALLKEPILSKFSPDPPILMKGLVACTGNQFCGQAIIETKARSLKITEEVQRQVSLTRPVRMHWTGCPNTCAQVQVADIGFMGCLTRDKDKKTVEGADVFLGGRIGSDSHLGEVYKKAVPCDELVPLIVDLLIKNFGAVPREREETED

SEQ ID NO: 6 - DNA, 1761 bp, Solanum lycopersicum
atggcatctttttctatcaaatttttggcaccttcattgccaaatccaactagattttccaagagtagtattgtcaagctcaatgcaactccgccgcagacagtggctgcggcggggcctccagaggttgctgctgagagactagaaccaagagttgaggaaaaagatggatattggatactaaaagagcagtttaggcaaggaattaatcctcaagagaaggtgaagattgagaaggaacctatgaagttgttcatggaaaatggtattgaggagttagctaagattccaattgaagagatagatcaatcaaagcttactaaggatgacattgatgttaggctcaagtggcttggcctcttccataggagaaagaatcaatatgggagattcatgatgaggttgaaacttccaaatggagtaacaacaagtgctcagactcgatatttggcgagtgtgataaggaaatatggagaggaaggatgtgctgatattacgacaaggcaaaattggcagattcgtggagtagtgctgcctgatgtgcctgagattctaaagggacttgaagaagttggcttgactagtttgcagagtggcatggataatgtcaggaatccagttggaaatcctctggctggaattgatcctgaagaaatagttgacacaagaccttacactaatttgctctcccaatttatcactggtaattcacgaggcaatccggctgtttctaacttgccaaggaagtggaatccgtgtgtagtagggtctcatgatctttatgagcaccctcatatcaatgatcttgcatacatgcctgccataaaagatggacgatttggattcaacctgcttgtgggagggttcttcagtgccaaaagatgtgatgaggcaattcctcttgatgcatgggttccagccgatgatgttgttccggtttgcaaggcaatactggaagcttttagagaccttgggttcagagggaacaggcagaagtgtagaatgatgtggttgatcgatgaactgggtgtagaaggattcagggcagaggtcgtaaagagaatgcctcagcaagagctagagagagcatctccggaagacttggttcagaaacaatgggaaagaagagattatcttggtgtacatccacagaaacaggaaggctatagctttattggtcttcacattccagtgggtcgtgtccaagcagacgacatggatgatctagctcgtttggctgatgagtacggctcaggagagctacggctgactgtggaacagaacattattattcccaacattgagaactcaaagattgacgcactgctaaaagagcctattttgagcaaattttcacctgatccacctattctcatgaaaggtttagtggcttgtactggtaaccagttttgtggacaagccattattgaaacgaaagctcgttccctgaagatcaccgaagaggttcaaaggcaagtatctctaacgaggccagtaaggatgcactggacaggctgcccaaatacgtgtgcacaagttcaagttgcagacattggattcatgggatgcctgactagagataaagacaagaagactgtggaaggcgccgatgttttcttaggaggcagaatagggagtgactcacatttgggtgaagtatacaagaaggcagttccttgtgatgaattagtaccacttattgtggacttacttattaagaactttggtgcagttccacgagaaagagaagaaacagaagat